European Patent Application EP 4 174 174 A1, published May 3, 2023. Title: TAILOR-MADE EXTREMOPHILIC FUNGAL LACCASES. Applicant: Consejo Superior de Investigaciones Científicas (CSIC). The sequence listing filed with the application follows.

SEQUENCE LISTING (52 sequences)

SEQ ID NO: 1 - protein, 496 aa, Artificial Sequence
  Engineered laccase RY2
SIGPVADLTISNGAVSPDGFSRQAILVNDVFPSPLITGNKGDRFQLNVIDNMTNHTMLKSTSIHWHGFFQHGTNWADGPAFVNQCPISTGHAFLYDFQVPDQAGTFWYHSHLSTQYCDGLRGPIVVYDPQDPHKSLYDVDDDSTVITLADWYHLAAKVGPAAPTADATLINGLGRSINTLNADLAVITVTKGKRYRFRLVSLSCDPSYTFSIDGHSLTVIEADGVNLKPQTVDSIQIFPAQRYSFVLNADQDVDNYWIRALPDSGTRNFDGGVNSAILRYEGAAPVEPTTSQTPSTQPLVESALTTLEGTAAPGNPTPGGVDLALNMAFGFAGGRFTINGASFTPPTVPVLLQILSGAQSAQDLLPSGSVYSLPANADIEISLPATSAAPGFPHPFHLHGHTFAVVRSAGSSTYNYANPVYRDVVNTGSPGDNVTIRFRTDNPGPWFLHCHIDPHLDAGFAVVMAEDTPDVAATNPVPQAWSDLCPIYDALDPSDL

SEQ ID NO: 2 - protein, 496 aa, Artificial Sequence
  Engineered laccase L1
SIGPVADLTISNGAVSPDGFSRQAILVNDVFPSPLITGNKGDRFQLNVIDNMTNHTMLKSTSIHWHGFFQHGTNWADGPAFVNQCPISTGHAFLYDFQVPDQAGTFWYHSHLSTQYCDGLRGPIVVYDPQDPHKSLYDVDDDSTVITLADWYHLAAKVGPAAPTADATLINGLGRSINTLNADLAVITVTKGKRYRFRLVSLSCDPSYTFSIDGHSLTVIEADGVNLKPQTVDSIQIFPAQRYSFVLNADQDVDNYWIRALPDSGTRNFDGGVNSAILRYEGAAPVEPTTSQTPSTQPLVESALTTLEGTAAPGNPTPGGVDLALNMAFGFAGGRFTINGASFTPPTVPVLLQILSGAQSAQDLLPSGSVYSLPANADIEISLPATSAAPGNPHPIHLHGHTFAVVRSAGSSTYNYANPVYRDVVNTGSPGDNVTIRFRTDNPGPWFLHCHIDPHLDAGFAVVMAEDTPDVAATNPVPQAWSDLCPIYDALDPSDL

SEQ ID NO: 3 - protein, 496 aa, Artificial Sequence
  Engineered laccase L2
SIGPVADLTISNGAVSPDGFSRQAILVNDVFPSPLITGNKGDRFQLNVIDNMTNHTMLKSTSIHWHGFFQHGTNWADGPAFVNQCPISTGHAFLYDFQVPDQAGTFWYHSHLSTQYCDGLRGPIVVYDPQDPHKSLYDVDDDSTVITLADWYHLAAKVGPAAPTADATLINGLGRSINTLNADLAVITVTKGKRYRFRLVSLSCDPSYTFSIDGHSLTVIEADGVNLKPQTVDSIQIFPAQRYSFVLNADQDVDNYWIRALPDSGTRNFDGGVNSAILRYEGAAPVEPTTSQTPSTQPLVESALTTLEGTAAPGNPTPGGVDLALNMAFGFAGGRFTINGASFTPPTVPVLLQILSGAQSAQDLLPSGSVYSLPANADIEISLPATSAAPGNPHPIHLHGHTFAVVRSAGSSTYNYANPVYRDVVNTGSPGDNVTIRFRTDNPGPWFLHCHIDPHLDAGMAVVMAEDTPDVAATNPVPQAWSDLCPIYDALDPSDL

SEQ ID NO: 4 - protein, 496 aa, Artificial Sequence
  Engineered laccase L3
SIGPVADLTISNGAVSPDGFSRQAILVNDVFPSPLITGNKGDRFQLNVIDNMTNHTMLKSTSIHWHGFFQHGTNWADGPAFVNQCPISTGHAFLYDFQVPDQAGTFWYHSHLSTQYCDGLRGPIVVYDPQDPHKSLYDVDDDSTVITLADWYHLAAKVGPAAPTADATLINGLGRSINTLNADLAVITVTKGKRYRFRLVSLSCDPSYTFSIDGHSLTVIEADGVNLKPQTVDSIQIFPAQRYSFVLNADQDVDNYWIRALPVSGTRNFDGGVNSAILRYEGAAPVEPTTSQTPSTQPLVESALTTLEGTAAPGNPTPGGVDLALNMAFGFAGGRFTINGASFTPPTVPVLLQILSGAQSAQDLLPSGSVYSLPANADIEISLPATSAAPGNPHPIHLHGHTFAVVRSAGSSTYNYANPVYRDVVNTGSPGDNVTIRFRTDNPGPWFLHCHIDPHLDAGMAVVMAEDTPDVAATNPVPQAWSDLCPIYDALDPSDL

SEQ ID NO: 5 - protein, 496 aa, Artificial Sequence
  Engineered laccase L4
SIGPVADLTISNGAVSPDGFSRQAILVNDVFPSPLITGNKGDRFQLNVIDNMTNHTMLKSTSIHWHGFFQHGTNWADGPAFVNQCPISTGHAFLYDFQVPDQAGTFWYHSHLSTQYCDGLRGPIVVYDPQDPHKSLYDVDDDSTVITLADWYHLAAKVGPAAPTADATLINGLGRSINTLNADLAVITVTKGKRYRFRLVSLSCDPSYTFSIDGHSLTVIEADGVNLKPQTVDSIQIFPAQRYSFVLNADQDVDNYWIRALPVSGTRNFDGGVNSAILRYEGAAPVEPTTSQTPSTQPLVESALTTLEGTAAPGNPTPGGVDLALNMAFGFAGGRFTINGASFTPPTVPVLLQILSGAQSAQDLLPSGSVYSLPANADIEISLPATSAAPGNPHPIHLHGHTFAVVRSAGSSTYNYANPVYRDVVNTGSPGDNVTIRFRTDNPGPWFLHCHIDPHLDLGMAVVMAEDTPDVAATNPVPQAWSDLCPIYDALDPSDL

SEQ ID NO: 6 - protein, 496 aa, Artificial Sequence
  Engineered laccase L5
SIGPVADLTISNGAVSPDGFSRQAILVNDVFPSPLITGNKGDRFQLNVIDNMTNHTMLKSTSIHWHGFFQHGTNWADGPAFVNQCPISTGHAFLYDFQVPDQAGTFWYHSHLSTQYCDGLRGPIVVYDPQDPHKSLYDVDDDSTVITLADWYHLAAKVGPAAPTADATLINGLGRSINTLNADLAVITVTKGKRYRFRLVSLSCDPSYTFSIDGHSLTVIEADGVNLKPQTVDSIQIFPAQRYSFVLNADQDVDNYWIRALPVSGTRNFDGGVNSAILRYEGAAPVEPTTSQTPSTQPLVESALTTLEGTAAPGNPTPGGVDLALNMAFGFAGGRFTINGASFTPPTVPVLLQILSGAQSAQDLLPSGSVYSLPANADIEISLPATSAAPGNPHPIHLHGHTFAVVRSAGSSTYNYANPVYRDTVNTGTPGDNVTIRFRTNNPGPWFLHCHIDPHLDLGMAVVMAEDTPDVAATNPVPQAWSDLCPIYDALDPSDL

SEQ ID NO: 7 - protein, 496 aa, Artificial Sequence
  Engineered laccase F392T-F396I
SIGPVADLTISNGAVSPDGFSRQAILVNDVFPSPLITGNKGDRFQLNVIDNMTNHTMLKSTSIHWHGFFQHGTNWADGPAFVNQCPISTGHAFLYDFQVPDQAGTFWYHSHLSTQYCDGLRGPIVVYDPQDPHKSLYDVDDDSTVITLADWYHLAAKVGPAAPTADATLINGLGRSINTLNADLAVITVTKGKRYRFRLVSLSCDPSYTFSIDGHSLTVIEADGVNLKPQTVDSIQIFPAQRYSFVLNADQDVDNYWIRALPDSGTRNFDGGVNSAILRYEGAAPVEPTTSQTPSTQPLVESALTTLEGTAAPGNPTPGGVDLALNMAFGFAGGRFTINGASFTPPTVPVLLQILSGAQSAQDLLPSGSVYSLPANADIEISLPATSAAPGTPHPIHLHGHTFAVVRSAGSSTYNYANPVYRDVVNTGSPGDNVTIRFRTDNPGPWFLHCHIDPHLDAGFAVVMAEDTPDVAATNPVPQAWSDLCPIYDALDPSDL

SEQ ID NO: 8 - protein, 496 aa, Artificial Sequence
  Engineered laccase F392T-F396I-F460M
SIGPVADLTISNGAVSPDGFSRQAILVNDVFPSPLITGNKGDRFQLNVIDNMTNHTMLKSTSIHWHGFFQHGTNWADGPAFVNQCPISTGHAFLYDFQVPDQAGTFWYHSHLSTQYCDGLRGPIVVYDPQDPHKSLYDVDDDSTVITLADWYHLAAKVGPAAPTADATLINGLGRSINTLNADLAVITVTKGKRYRFRLVSLSCDPSYTFSIDGHSLTVIEADGVNLKPQTVDSIQIFPAQRYSFVLNADQDVDNYWIRALPDSGTRNFDGGVNSAILRYEGAAPVEPTTSQTPSTQPLVESALTTLEGTAAPGNPTPGGVDLALNMAFGFAGGRFTINGASFTPPTVPVLLQILSGAQSAQDLLPSGSVYSLPANADIEISLPATSAAPGTPHPIHLHGHTFAVVRSAGSSTYNYANPVYRDVVNTGSPGDNVTIRFRTDNPGPWFLHCHIDPHLDAGMAVVMAEDTPDVAATNPVPQAWSDLCPIYDALDPSDL

SEQ ID NO: 9 - protein, 496 aa, Artificial Sequence
  Engineered laccase F392T-F396I-F460M-D263V
SIGPVADLTISNGAVSPDGFSRQAILVNDVFPSPLITGNKGDRFQLNVIDNMTNHTMLKSTSIHWHGFFQHGTNWADGPAFVNQCPISTGHAFLYDFQVPDQAGTFWYHSHLSTQYCDGLRGPIVVYDPQDPHKSLYDVDDDSTVITLADWYHLAAKVGPAAPTADATLINGLGRSINTLNADLAVITVTKGKRYRFRLVSLSCDPSYTFSIDGHSLTVIEADGVNLKPQTVDSIQIFPAQRYSFVLNADQDVDNYWIRALPVSGTRNFDGGVNSAILRYEGAAPVEPTTSQTPSTQPLVESALTTLEGTAAPGNPTPGGVDLALNMAFGFAGGRFTINGASFTPPTVPVLLQILSGAQSAQDLLPSGSVYSLPANADIEISLPATSAAPGTPHPIHLHGHTFAVVRSAGSSTYNYANPVYRDVVNTGSPGDNVTIRFRTDNPGPWFLHCHIDPHLDAGMAVVMAEDTPDVAATNPVPQAWSDLCPIYDALDPSDL

SEQ ID NO: 10 - protein, 496 aa, Artificial Sequence
  Engineered laccase F392T-F396I-F460M-D263V-A458L
SIGPVADLTISNGAVSPDGFSRQAILVNDVFPSPLITGNKGDRFQLNVIDNMTNHTMLKSTSIHWHGFFQHGTNWADGPAFVNQCPISTGHAFLYDFQVPDQAGTFWYHSHLSTQYCDGLRGPIVVYDPQDPHKSLYDVDDDSTVITLADWYHLAAKVGPAAPTADATLINGLGRSINTLNADLAVITVTKGKRYRFRLVSLSCDPSYTFSIDGHSLTVIEADGVNLKPQTVDSIQIFPAQRYSFVLNADQDVDNYWIRALPVSGTRNFDGGVNSAILRYEGAAPVEPTTSQTPSTQPLVESALTTLEGTAAPGNPTPGGVDLALNMAFGFAGGRFTINGASFTPPTVPVLLQILSGAQSAQDLLPSGSVYSLPANADIEISLPATSAAPGTPHPIHLHGHTFAVVRSAGSSTYNYANPVYRDVVNTGSPGDNVTIRFRTDNPGPWFLHCHIDPHLDLGMAVVMAEDTPDVAATNPVPQAWSDLCPIYDALDPSDL

SEQ ID NO: 11 - protein, 496 aa, Artificial Sequence
  Engineered laccase F392T-F396I-F460M-D263V-A458L-V424T-S429T-D441N
SIGPVADLTISNGAVSPDGFSRQAILVNDVFPSPLITGNKGDRFQLNVIDNMTNHTMLKSTSIHWHGFFQHGTNWADGPAFVNQCPISTGHAFLYDFQVPDQAGTFWYHSHLSTQYCDGLRGPIVVYDPQDPHKSLYDVDDDSTVITLADWYHLAAKVGPAAPTADATLINGLGRSINTLNADLAVITVTKGKRYRFRLVSLSCDPSYTFSIDGHSLTVIEADGVNLKPQTVDSIQIFPAQRYSFVLNADQDVDNYWIRALPVSGTRNFDGGVNSAILRYEGAAPVEPTTSQTPSTQPLVESALTTLEGTAAPGNPTPGGVDLALNMAFGFAGGRFTINGASFTPPTVPVLLQILSGAQSAQDLLPSGSVYSLPANADIEISLPATSAAPGTPHPIHLHGHTFAVVRSAGSSTYNYANPVYRDTVNTGTPGDNVTIRFRTNNPGPWFLHCHIDPHLDLGMAVVMAEDTPDVAATNPVPQAWSDLCPIYDALDPSDL

SEQ ID NO: 12 - protein, 496 aa, Artificial Sequence
  Engineered laccase F392T-F396I-F460M-D263A
SIGPVADLTISNGAVSPDGFSRQAILVNDVFPSPLITGNKGDRFQLNVIDNMTNHTMLKSTSIHWHGFFQHGTNWADGPAFVNQCPISTGHAFLYDFQVPDQAGTFWYHSHLSTQYCDGLRGPIVVYDPQDPHKSLYDVDDDSTVITLADWYHLAAKVGPAAPTADATLINGLGRSINTLNADLAVITVTKGKRYRFRLVSLSCDPSYTFSIDGHSLTVIEADGVNLKPQTVDSIQIFPAQRYSFVLNADQDVDNYWIRALPASGTRNFDGGVNSAILRYEGAAPVEPTTSQTPSTQPLVESALTTLEGTAAPGNPTPGGVDLALNMAFGFAGGRFTINGASFTPPTVPVLLQILSGAQSAQDLLPSGSVYSLPANADIEISLPATSAAPGTPHPIHLHGHTFAVVRSAGSSTYNYANPVYRDVVNTGSPGDNVTIRFRTDNPGPWFLHCHIDPHLDAGMAVVMAEDTPDVAATNPVPQAWSDLCPIYDALDPSDL

SEQ ID NO: 13 - protein, 496 aa, Artificial Sequence
  Engineered laccase F392T-F396I-F460M-D263A-A458L
SIGPVADLTISNGAVSPDGFSRQAILVNDVFPSPLITGNKGDRFQLNVIDNMTNHTMLKSTSIHWHGFFQHGTNWADGPAFVNQCPISTGHAFLYDFQVPDQAGTFWYHSHLSTQYCDGLRGPIVVYDPQDPHKSLYDVDDDSTVITLADWYHLAAKVGPAAPTADATLINGLGRSINTLNADLAVITVTKGKRYRFRLVSLSCDPSYTFSIDGHSLTVIEADGVNLKPQTVDSIQIFPAQRYSFVLNADQDVDNYWIRALPASGTRNFDGGVNSAILRYEGAAPVEPTTSQTPSTQPLVESALTTLEGTAAPGNPTPGGVDLALNMAFGFAGGRFTINGASFTPPTVPVLLQILSGAQSAQDLLPSGSVYSLPANADIEISLPATSAAPGTPHPIHLHGHTFAVVRSAGSSTYNYANPVYRDVVNTGSPGDNVTIRFRTDNPGPWFLHCHIDPHLDLGMAVVMAEDTPDVAATNPVPQAWSDLCPIYDALDPSDL

SEQ ID NO: 14 - protein, 496 aa, Artificial Sequence
  Engineered laccase F392T-F396I-F460M-D263A-A458L-V424T-S429T-D441N
SIGPVADLTISNGAVSPDGFSRQAILVNDVFPSPLITGNKGDRFQLNVIDNMTNHTMLKSTSIHWHGFFQHGTNWADGPAFVNQCPISTGHAFLYDFQVPDQAGTFWYHSHLSTQYCDGLRGPIVVYDPQDPHKSLYDVDDDSTVITLADWYHLAAKVGPAAPTADATLINGLGRSINTLNADLAVITVTKGKRYRFRLVSLSCDPSYTFSIDGHSLTVIEADGVNLKPQTVDSIQIFPAQRYSFVLNADQDVDNYWIRALPASGTRNFDGGVNSAILRYEGAAPVEPTTSQTPSTQPLVESALTTLEGTAAPGNPTPGGVDLALNMAFGFAGGRFTINGASFTPPTVPVLLQILSGAQSAQDLLPSGSVYSLPANADIEISLPATSAAPGTPHPIHLHGHTFAVVRSAGSSTYNYANPVYRDTVNTGTPGDNVTIRFRTNNPGPWFLHCHIDPHLDLGMAVVMAEDTPDVAATNPVPQAWSDLCPIYDALDPSDL

SEQ ID NO: 15 - protein, 496 aa, Artificial Sequence
  Engineered laccase F392T-F396I-F460M-D263G
SIGPVADLTISNGAVSPDGFSRQAILVNDVFPSPLITGNKGDRFQLNVIDNMTNHTMLKSTSIHWHGFFQHGTNWADGPAFVNQCPISTGHAFLYDFQVPDQAGTFWYHSHLSTQYCDGLRGPIVVYDPQDPHKSLYDVDDDSTVITLADWYHLAAKVGPAAPTADATLINGLGRSINTLNADLAVITVTKGKRYRFRLVSLSCDPSYTFSIDGHSLTVIEADGVNLKPQTVDSIQIFPAQRYSFVLNADQDVDNYWIRALPGSGTRNFDGGVNSAILRYEGAAPVEPTTSQTPSTQPLVESALTTLEGTAAPGNPTPGGVDLALNMAFGFAGGRFTINGASFTPPTVPVLLQILSGAQSAQDLLPSGSVYSLPANADIEISLPATSAAPGTPHPIHLHGHTFAVVRSAGSSTYNYANPVYRDVVNTGSPGDNVTIRFRTDNPGPWFLHCHIDPHLDAGMAVVMAEDTPDVAATNPVPQAWSDLCPIYDALDPSDL

SEQ ID NO: 16 - protein, 496 aa, Artificial Sequence
  Engineered laccase F392T-F396I-F460M-D263G-A458L
SIGPVADLTISNGAVSPDGFSRQAILVNDVFPSPLITGNKGDRFQLNVIDNMTNHTMLKSTSIHWHGFFQHGTNWADGPAFVNQCPISTGHAFLYDFQVPDQAGTFWYHSHLSTQYCDGLRGPIVVYDPQDPHKSLYDVDDDSTVITLADWYHLAAKVGPAAPTADATLINGLGRSINTLNADLAVITVTKGKRYRFRLVSLSCDPSYTFSIDGHSLTVIEADGVNLKPQTVDSIQIFPAQRYSFVLNADQDVDNYWIRALPGSGTRNFDGGVNSAILRYEGAAPVEPTTSQTPSTQPLVESALTTLEGTAAPGNPTPGGVDLALNMAFGFAGGRFTINGASFTPPTVPVLLQILSGAQSAQDLLPSGSVYSLPANADIEISLPATSAAPGTPHPIHLHGHTFAVVRSAGSSTYNYANPVYRDVVNTGSPGDNVTIRFRTDNPGPWFLHCHIDPHLDLGMAVVMAEDTPDVAATNPVPQAWSDLCPIYDALDPSDL

SEQ ID NO: 17 - protein, 496 aa, Artificial Sequence
  Engineered laccase F392T-F396I-F460M-D263G-A458L-V424T-S429T-D441N
SIGPVADLTISNGAVSPDGFSRQAILVNDVFPSPLITGNKGDRFQLNVIDNMTNHTMLKSTSIHWHGFFQHGTNWADGPAFVNQCPISTGHAFLYDFQVPDQAGTFWYHSHLSTQYCDGLRGPIVVYDPQDPHKSLYDVDDDSTVITLADWYHLAAKVGPAAPTADATLINGLGRSINTLNADLAVITVTKGKRYRFRLVSLSCDPSYTFSIDGHSLTVIEADGVNLKPQTVDSIQIFPAQRYSFVLNADQDVDNYWIRALPGSGTRNFDGGVNSAILRYEGAAPVEPTTSQTPSTQPLVESALTTLEGTAAPGNPTPGGVDLALNMAFGFAGGRFTINGASFTPPTVPVLLQILSGAQSAQDLLPSGSVYSLPANADIEISLPATSAAPGTPHPIHLHGHTFAVVRSAGSSTYNYANPVYRDTVNTGTPGDNVTIRFRTNNPGPWFLHCHIDPHLDLGMAVVMAEDTPDVAATNPVPQAWSDLCPIYDALDPSDL

SEQ ID NO: 18 - protein, 91 aa, Artificial Sequence
  Signal peptide RY2-L4
MRFPSIFTDVLFAASSALATPVNTTTEDETAHIPAEAVIGYSDLEGDSDVAVLPFSNGTNNRLLFINTTIASIAAKEEGVSLEKRETEAEF

SEQ ID NO: 19 - protein, 91 aa, Artificial Sequence
  Signal peptide L5
MRFPSIFTDVLFAASSALATPVNTTTEDETAQIPAEAVIGYSDLEGDFDVAVLPFSNSTNNGLLFINTTIASIAAKEEGVSLEKRTNEAEF

SEQ ID NO: 20 - protein, 496 aa, Artificial Sequence
  Engineered laccase F392N-F396I-F460M-D263A
SIGPVADLTISNGAVSPDGFSRQAILVNDVFPSPLITGNKGDRFQLNVIDNMTNHTMLKSTSIHWHGFFQHGTNWADGPAFVNQCPISTGHAFLYDFQVPDQAGTFWYHSHLSTQYCDGLRGPIVVYDPQDPHKSLYDVDDDSTVITLADWYHLAAKVGPAAPTADATLINGLGRSINTLNADLAVITVTKGKRYRFRLVSLSCDPSYTFSIDGHSLTVIEADGVNLKPQTVDSIQIFPAQRYSFVLNADQDVDNYWIRALPASGTRNFDGGVNSAILRYEGAAPVEPTTSQTPSTQPLVESALTTLEGTAAPGNPTPGGVDLALNMAFGFAGGRFTINGASFTPPTVPVLLQILSGAQSAQDLLPSGSVYSLPANADIEISLPATSAAPGNPHPIHLHGHTFAVVRSAGSSTYNYANPVYRDVVNTGSPGDNVTIRFRTDNPGPWFLHCHIDPHLDAGMAVVMAEDTPDVAATNPVPQAWSDLCPIYDALDPSDL

SEQ ID NO: 21 - protein, 496 aa, Artificial Sequence
  Engineered laccase F392N-F396I-F460M-D263A-A458L
SIGPVADLTISNGAVSPDGFSRQAILVNDVFPSPLITGNKGDRFQLNVIDNMTNHTMLKSTSIHWHGFFQHGTNWADGPAFVNQCPISTGHAFLYDFQVPDQAGTFWYHSHLSTQYCDGLRGPIVVYDPQDPHKSLYDVDDDSTVITLADWYHLAAKVGPAAPTADATLINGLGRSINTLNADLAVITVTKGKRYRFRLVSLSCDPSYTFSIDGHSLTVIEADGVNLKPQTVDSIQIFPAQRYSFVLNADQDVDNYWIRALPASGTRNFDGGVNSAILRYEGAAPVEPTTSQTPSTQPLVESALTTLEGTAAPGNPTPGGVDLALNMAFGFAGGRFTINGASFTPPTVPVLLQILSGAQSAQDLLPSGSVYSLPANADIEISLPATSAAPGNPHPIHLHGHTFAVVRSAGSSTYNYANPVYRDVVNTGSPGDNVTIRFRTDNPGPWFLHCHIDPHLDLGMAVVMAEDTPDVAATNPVPQAWSDLCPIYDALDPSDL

SEQ ID NO: 22 - protein, 496 aa, Artificial Sequence
  Engineered laccase F392N-F396I-F460M-D263A-A458L- V424T-S429T-D441N
SIGPVADLTISNGAVSPDGFSRQAILVNDVFPSPLITGNKGDRFQLNVIDNMTNHTMLKSTSIHWHGFFQHGTNWADGPAFVNQCPISTGHAFLYDFQVPDQAGTFWYHSHLSTQYCDGLRGPIVVYDPQDPHKSLYDVDDDSTVITLADWYHLAAKVGPAAPTADATLINGLGRSINTLNADLAVITVTKGKRYRFRLVSLSCDPSYTFSIDGHSLTVIEADGVNLKPQTVDSIQIFPAQRYSFVLNADQDVDNYWIRALPASGTRNFDGGVNSAILRYEGAAPVEPTTSQTPSTQPLVESALTTLEGTAAPGNPTPGGVDLALNMAFGFAGGRFTINGASFTPPTVPVLLQILSGAQSAQDLLPSGSVYSLPANADIEISLPATSAAPGNPHPIHLHGHTFAVVRSAGSSTYNYANPVYRDTVNTGTPGDNVTIRFRTNNPGPWFLHCHIDPHLDLGMAVVMAEDTPDVAATNPVPQAWSDLCPIYDALDPSDL

SEQ ID NO: 23 - protein, 496 aa, Artificial Sequence; identical to SEQ ID NO: 20
  Engineered laccase F392N-F396I-F460M-D263G

SEQ ID NO: 24 - protein, 496 aa, Artificial Sequence; identical to SEQ ID NO: 21
  Engineered laccase F392N-F396I-F460M-D263G-A458L

SEQ ID NO: 25 - protein, 496 aa, Artificial Sequence; identical to SEQ ID NO: 22
  Engineered laccase F392N-F396I-F460M-D263G-A458L- V424T-S429T-D441N

SEQ ID NO: 26 - DNA, 1491 bp, Artificial Sequence
  Engineered laccase RY2
agcattgggccagtcgcagacctcaccatctccaacggtgctgtcagtcccgatggtttctctcggcaggccatcctggtcaacgacgtcttccccagtcccctcattacggggaacaagggtgatcgtttccaactcaatgtcatcgacaacatgaccaaccacaccatgttgaagtccaccagtatccattggcacggcttcttccagcacggcaccaactgggccgacggccccgccttcgtgaaccagtgcccgatttctaccgggcatgcgttcctttacgacttccaggtccctgaccaagctggtactttctggtaccacagtcacttgtccactcaatactgtgacggtctcaggggtccgattgttgtctatgaccctcaagatccccacaagagcctttacgatgttgatgacgactccactgtaatcactctcgcggattggtaccacttggctgccaaagtcggcccggcggccccgactgccgatgctactcttatcaacggcctcggtcgcagcatcaacacgctcaacgccgatttggctgtcatcacggtcacgaagggcaagcgctatcgcttccgcctggtgtcgctgtcatgcgacccgtcttacacgttcagcattgatggtcactctctgaccgtcatcgaggcggacggcgtgaatctcaagccccagactgtcgactccatccagatcttccctgcccagcgatactcgtttgtgctcaacgcagatcaggatgtggacaactactggatccgtgcccttcccgattccgggaccaggaacttcgacggcggcgttaactccgccatccttcgctacgaaggtgctgcgcccgttgagcccaccacgagccagacgccgtcgacgcagcctttggtggagtccgccctgaccactctcgaaggcaccgctgcgcccggcaacccgacccctggcggtgtcgacctggctctcaacatggctttcggctttgccggcggcaggttcaccatcaacggcgcgagcttcaccccgcccaccgtccccgtcctcctgcagatcctgagcggcgcgcagtcggcgcaggacctcctcccctctggaagtgtatactcgctccctgcgaacgcggacattgagatctccctccccgccacctccgccgcccccggctttccgcacccctttcacttgcacgggcacaccttcgccgtcgtgcgcagcgccggctcgtcgacgtacaactacgcgaacccggtctaccgcgacgtcgtcaacacgggctcgcccggggacaacgtcacgatccggttcaggacggacaacccaggcccgtggttcctccactgccacattgaccctcacctcgacgccggctttgctgtagtcatggccgaggacactcccgacgtcgccgctacgaacccggtcccgcaagcatggtcggacttgtgccccatctatgatgcacttgaccccagcgacctctga

SEQ ID NO: 27 - DNA, 1491 bp, Artificial Sequence
  Engineered laccase L1
agcattgggccagtcgcagacctcaccatctccaacggtgctgtcagtcccgatggtttctctcggcaggccatcctggtcaacgacgtcttccccagtcccctcattacggggaacaagggtgatcgtttccaactcaatgtcatcgacaacatgaccaaccacaccatgttgaagtccaccagtatccattggcacggcttcttccagcacggcaccaactgggccgacggccccgccttcgtgaaccagtgcccgatttctaccgggcatgcgttcctttacgacttccaggtccctgaccaagctggtactttctggtaccacagtcacttgtccactcaatactgtgacggtctcaggggtccgattgttgtctatgaccctcaagatccccacaagagcctttacgatgttgatgacgactccactgtaatcactctcgcggattggtaccacttggctgccaaagtcggcccggcggccccgactgccgatgctactcttatcaacggcctcggtcgcagcatcaacacgctcaacgccgatttggctgtcatcacggtcacgaagggcaagcgctatcgcttccgcctggtgtcgctgtcatgcgacccgtcttacacgttcagcattgatggtcactctctgaccgtcatcgaggcggacggcgtgaatctcaagccccagactgtcgactccatccagatcttccctgcccagcgatactcgtttgtgctcaacgcagatcaggatgtggacaactactggatccgtgcccttcccgattccgggaccaggaacttcgacggcggcgttaactccgccatccttcgctacgaaggtgctgcgcccgttgagcccaccacgagccagacgccgtcgacgcagcctttggtggagtccgccctgaccactctcgaaggcaccgctgcgcccggcaacccgacccctggcggtgtcgacctggctctcaacatggctttcggctttgccggcggcaggttcaccatcaacggcgcgagcttcaccccgcccaccgtccccgtcctcctgcagatcctgagcggcgcgcagtcggcgcaggacctcctcccctctggaagtgtatactcgctccctgcgaacgcggacattgagatctccctccccgccacctccgccgcccccggcaatccgcaccccatccacttgcacgggcacaccttcgccgtcgtgcgcagcgccggctcgtcgacgtacaactacgcgaacccggtctaccgcgacgtcgtcaacacgggctcgcccggggacaacgtcacgatccggttcaggacggacaacccaggcccgtggttcctccactgccacattgaccctcacctcgacgccggctttgctgtagtcatggccgaggacactcccgacgtcgccgctacgaacccggtcccgcaagcatggtcggacttgtgccccatctatgatgcacttgaccccagcgacctctga

SEQ ID NO: 28 - DNA, 1491 bp, Artificial Sequence
  Engineered laccase L2
agcattgggccagtcgcagacctcaccatctccaacggtgctgtcagtcccgatggtttctctcggcaggccatcctggtcaacgacgtcttccccagtcccctcattacggggaacaagggtgatcgtttccaactcaatgtcatcgacaacatgaccaaccacaccatgttgaagtccaccagtatccattggcacggcttcttccagcacggcaccaactgggccgacggccccgccttcgtgaaccagtgcccgatttctaccgggcatgcgttcctttacgacttccaggtccctgaccaagctggtactttctggtaccacagtcacttgtccactcaatactgtgacggtctcaggggtccgattgttgtctatgaccctcaagatccccacaagagcctttacgatgttgatgacgactccactgtaatcactctcgcggattggtaccacttggctgccaaagtcggcccggcggccccgactgccgatgctactcttatcaacggcctcggtcgcagcatcaacacgctcaacgccgatttggctgtcatcacggtcacgaagggcaagcgctatcgcttccgcctggtgtcgctgtcatgcgacccgtcttacacgttcagcattgatggtcactctctgaccgtcatcgaggcggacggcgtgaatctcaagccccagactgtcgactccatccagatcttccctgcccagcgatactcgtttgtgctcaacgcagatcaggatgtggacaactactggatccgtgcccttcccgattccgggaccaggaacttcgacggcggcgttaactccgccatccttcgctacgaaggtgctgcgcccgttgagcccaccacgagccagacgccgtcgacgcagcctttggtggagtccgccctgaccactctcgaaggcaccgctgcgcccggcaacccgacccctggcggtgtcgacctggctctcaacatggctttcggctttgccggcggcaggttcaccatcaacggcgcgagcttcaccccgcccaccgtccccgtcctcctgcagatcctgagcggcgcgcagtcggcgcaggacctcctcccctctggaagtgtatactcgctccctgcgaacgcggacattgagatctccctccccgccacctccgccgcccccggcaatccgcaccccatccacttgcacgggcacaccttcgccgtcgtgcgcagcgccggctcgtcgacgtacaactacgcgaacccggtctaccgcgacgtcgtcaacacgggctcgcccggggacaacgtcacgatccggttcaggacggacaacccaggcccgtggttcctccactgccacattgaccctcacctcgacgccggcatggctgtagtcatggccgaggacactcccgacgtcgccgctacgaacccggtcccgcaagcatggtcggacttgtgccccatctatgatgcacttgaccccagcgacctctga

SEQ ID NO: 29 - DNA, 1491 bp, Artificial Sequence
  Engineered laccase L3
agcattgggccagtcgcagacctcaccatctccaacggtgctgtcagtcccgatggtttctctcggcaggccatcctggtcaacgacgtcttccccagtcccctcattacggggaacaagggtgatcgtttccaactcaatgtcatcgacaacatgaccaaccacaccatgttgaagtccaccagtatccattggcacggcttcttccagcacggcaccaactgggccgacggccccgccttcgtgaaccagtgcccgatttctaccgggcatgcgttcctttacgacttccaggtccctgaccaagctggtactttctggtaccacagtcacttgtccactcaatactgtgacggtctcaggggtccgattgttgtctatgaccctcaagatccccacaagagcctttacgatgttgatgacgactccactgtaatcactctcgcggattggtaccacttggctgccaaagtcggcccggcggccccgactgccgatgctactcttatcaacggcctcggtcgcagcatcaacacgctcaacgccgatttggctgtcatcacggtcacgaagggcaagcgctatcgcttccgcctggtgtcgctgtcatgcgacccgtcttacacgttcagcattgatggtcactctctgaccgtcatcgaggcggacggcgtgaatctcaagccccagactgtcgactccatccagatcttccctgcccagcgatactcgtttgtgctcaacgcagatcaggatgtggacaactactggatccgtgcccttcccgtttccgggaccaggaacttcgacggcggcgttaactccgccatccttcgctacgaaggtgctgcgcccgttgagcccaccacgagccagacgccgtcgacgcagcctttggtggagtccgccctgaccactctcgaaggcaccgctgcgcccggcaacccgacccctggcggtgtcgacctggctctcaacatggctttcggctttgccggcggcaggttcaccatcaacggcgcgagcttcaccccgcccaccgtccccgtcctcctgcagatcctgagcggcgcgcagtcggcgcaggacctcctcccctctggaagtgtatactcgctccctgcgaacgcggacattgagatctccctccccgccacctccgccgcccccggcaatccgcaccccatccacttgcacgggcacaccttcgccgtcgtgcgcagcgccggctcgtcgacgtacaactacgcgaacccggtctaccgcgacgtcgtcaacacgggctcgcccggggacaacgtcacgatccggttcaggacggacaacccaggcccgtggttcctccactgccacattgaccctcacctcgacgccggcatggctgtagtcatggccgaggacactcccgacgtcgccgctacgaacccggtcccgcaagcatggtcggacttgtgccccatctatgatgcacttgaccccagcgacctctga

SEQ ID NO: 30 - DNA, 1491 bp, Artificial Sequence
  Engineered laccase L4
agcattgggccagtcgcagacctcaccatctccaacggtgctgtcagtcccgatggtttctctcggcaggccatcctggtcaacgacgtcttccccagtcccctcattacggggaacaagggtgatcgtttccaactcaatgtcatcgacaacatgaccaaccacaccatgttgaagtccaccagtatccattggcacggcttcttccagcacggcaccaactgggccgacggccccgccttcgtgaaccagtgcccgatttctaccgggcatgcgttcctttacgacttccaggtccctgaccaagctggtactttctggtaccacagtcacttgtccactcaatactgtgacggtctcaggggtccgattgttgtctatgaccctcaagatccccacaagagcctttacgatgttgatgacgactccactgtaatcactctcgcggattggtaccacttggctgccaaagtcggcccggcggccccgactgccgatgctactcttatcaacggcctcggtcgcagcatcaacacgctcaacgccgatttggctgtcatcacggtcacgaagggcaagcgctatcgcttccgcctggtgtcgctgtcatgcgacccgtcttacacgttcagcattgatggtcactctctgaccgtcatcgaggcggacggcgtgaatctcaagccccagactgtcgactccatccagatcttccctgcccagcgatactcgtttgtgctcaacgcagatcaggatgtggacaactactggatccgtgcccttcccgtttccgggaccaggaacttcgacggcggcgttaactccgccatccttcgctacgaaggtgctgcgcccgttgagcccaccacgagccagacgccgtcgacgcagcctttggtggagtccgccctgaccactctcgaaggcaccgctgcgcccggcaacccgacccctggcggtgtcgacctggctctcaacatggctttcggctttgccggcggcaggttcaccatcaacggcgcgagcttcaccccgcccaccgtccccgtcctcctgcagatcctgagcggcgcgcagtcggcgcaggacctcctcccctctggaagtgtatactcgctccctgcgaacgcggacattgagatctccctccccgccacctccgccgcccccggcaatccgcaccccatccacttgcacgggcacaccttcgccgtcgtgcgcagcgccggctcgtcgacgtacaactacgcgaacccggtctaccgcgacgtcgtcaacacgggctcgcccggggacaacgtcacgatccggttcaggacggacaacccaggcccgtggttcctccactgccacattgaccctcacctcgacctaggcatggctgtagtcatggccgaggacactcccgacgtcgccgctacgaacccggtcccgcaagcatggtcggacttgtgccccatctatgatgcacttgaccccagcgacctctga

SEQ ID NO: 31 - DNA, 1491 bp, Artificial Sequence
  Engineered laccase L5
agcattgggccagtcgcagacctcaccatctccaacggtgctgtcagtcccgatggtttctctcggcaggccatcctggtcaacgacgtcttccccagtcccctcattacggggaacaagggtgatcgtttccaactcaatgtcatcgacaacatgaccaaccacaccatgttgaagtccaccagtatccattggcacggcttcttccagcacggcaccaactgggccgacggccccgccttcgtgaaccagtgcccgatttctaccgggcatgcgttcctttacgacttccaggtccctgaccaagctggtactttctggtaccacagtcacttgtccactcaatactgtgacggtctcaggggtccgattgttgtctatgaccctcaagatccccacaagagcctttacgatgttgatgacgactccactgtaatcactctcgcggattggtaccacttggctgccaaagtcggcccggcggccccgactgccgatgctactcttatcaacggcctcggtcgcagcatcaacacgctcaacgccgatttggctgtcatcacggtcacgaagggcaagcgctatcgcttccgcctggtgtcgctgtcatgcgacccgtcttacacgttcagcattgatggtcactctctgaccgtcatcgaggcggacggcgtgaatctcaagccccagactgtcgactccatccagatcttccctgcccagcgatactcgtttgtgctcaacgcagatcaggatgtggacaactactggatccgtgcccttcccgtttccgggaccaggaacttcgacggcggcgttaactccgccatccttcgctacgaaggtgctgcgcccgttgagcccaccacgagccagacgccgtcgacgcagcctttggtggagtccgccctgaccactctcgaaggcaccgctgcgcccggcaacccgacccctggcggtgtcgacctggctctcaacatggctttcggctttgccggcggcaggttcaccatcaacggcgcgagcttcaccccgcccaccgtccccgtcctcctgcagatcctgagcggcgcgcagtcggcgcaggacctcctcccctctggaagtgtatactcgctccctgcgaacgcggacattgagatctccctccccgccacctccgccgcccccggcaatccgcaccccatccacttgcacgggcacaccttcgccgtcgtgcgcagcgccggctcgtcgacgtacaactacgcgaacccggtctaccgcgacactgtcaacacgggcactcccggggacaacgtcacgatccggttcaggacgaataacccaggcccgtggttcctccactgccacattgaccctcacctcgacctaggcatggctgtagtcatggccgaggacactcccgacgtcgccgctacgaacccggtcccgcaagcatggtcggacttgtgccccatctatgatgcacttgaccccagcgacctctga

SEQ ID NO: 32 - DNA, 1491 bp, Artificial Sequence
  Engineered laccase F392T-F396I
agcattgggccagtcgcagacctcaccatctccaacggtgctgtcagtcccgatggtttctctcggcaggccatcctggtcaacgacgtcttccccagtcccctcattacggggaacaagggtgatcgtttccaactcaatgtcatcgacaacatgaccaaccacaccatgttgaagtccaccagtatccattggcacggcttcttccagcacggcaccaactgggccgacggccccgccttcgtgaaccagtgcccgatttctaccgggcatgcgttcctttacgacttccaggtccctgaccaagctggtactttctggtaccacagtcacttgtccactcaatactgtgacggtctcaggggtccgattgttgtctatgaccctcaagatccccacaagagcctttacgatgttgatgacgactccactgtaatcactctcgcggattggtaccacttggctgccaaagtcggcccggcggccccgactgccgatgctactcttatcaacggcctcggtcgcagcatcaacacgctcaacgccgatttggctgtcatcacggtcacgaagggcaagcgctatcgcttccgcctggtgtcgctgtcatgcgacccgtcttacacgttcagcattgatggtcactctctgaccgtcatcgaggcggacggcgtgaatctcaagccccagactgtcgactccatccagatcttccctgcccagcgatactcgtttgtgctcaacgcagatcaggatgtggacaactactggatccgtgcccttcccgattccgggaccaggaacttcgacggcggcgttaactccgccatccttcgctacgaaggtgctgcgcccgttgagcccaccacgagccagacgccgtcgacgcagcctttggtggagtccgccctgaccactctcgaaggcaccgctgcgcccggcaacccgacccctggcggtgtcgacctggctctcaacatggctttcggctttgccggcggcaggttcaccatcaacggcgcgagcttcaccccgcccaccgtccccgtcctcctgcagatcctgagcggcgcgcagtcggcgcaggacctcctcccctctggaagtgtatactcgctccctgcgaacgcggacattgagatctccctccccgccacctccgccgcccccggcacuccgcaccccatccacttgcacgggcacaccttcgccgtcgtgcgcagcgccggctcgtcgacgtacaactacgcgaacccggtctaccgcgacgtcgtcaacacgggctcgcccggggacaacgtcacgatccggttcaggacggacaacccaggcccgtggttcctccactgccacattgaccctcacctcgacgccggctttgctgtagtcatggccgaggacactcccgacgtcgccgctacgaacccggtcccgcaagcatggtcggacttgtgccccatctatgatgcacttgaccccagcgacctctga

SEQ ID NO: 33 - DNA, 1491 bp, Artificial Sequence
  Engineered laccase F392T-F396I-F460M
agcattgggccagtcgcagacctcaccatctccaacggtgctgtcagtcccgatggtttctctcggcaggccatcctggtcaacgacgtcttccccagtcccctcattacggggaacaagggtgatcgtttccaactcaatgtcatcgacaacatgaccaaccacaccatgttgaagtccaccagtatccattggcacggcttcttccagcacggcaccaactgggccgacggccccgccttcgtgaaccagtgcccgatttctaccgggcatgcgttcctttacgacttccaggtccctgaccaagctggtactttctggtaccacagtcacttgtccactcaatactgtgacggtctcaggggtccgattgttgtctatgaccctcaagatccccacaagagcctttacgatgttgatgacgactccactgtaatcactctcgcggattggtaccacttggctgccaaagtcggcccggcggccccgactgccgatgctactcttatcaacggcctcggtcgcagcatcaacacgctcaacgccgatttggctgtcatcacggtcacgaagggcaagcgctatcgcttccgcctggtgtcgctgtcatgcgacccgtcttacacgttcagcattgatggtcactctctgaccgtcatcgaggcggacggcgtgaatctcaagccccagactgtcgactccatccagatcttccctgcccagcgatactcgtttgtgctcaacgcagatcaggatgtggacaactactggatccgtgcccttcccgattccgggaccaggaacttcgacggcggcgttaactccgccatccttcgctacgaaggtgctgcgcccgttgagcccaccacgagccagacgccgtcgacgcagcctttggtggagtccgccctgaccactctcgaaggcaccgctgcgcccggcaacccgacccctggcggtgtcgacctggctctcaacatggctttcggctttgccggcggcaggttcaccatcaacggcgcgagcttcaccccgcccaccgtccccgtcctcctgcagatcctgagcggcgcgcagtcggcgcaggacctcctcccctctggaagtgtatactcgctccctgcgaacgcggacattgagatctccctccccgccacctccgccgcccccggcacuccgcaccccatccacttgcacgggcacaccttcgccgtcgtgcgcagcgccggctcgtcgacgtacaactacgcgaacccggtctaccgcgacgtcgtcaacacgggctcgcccggggacaacgtcacgatccggttcaggacggacaacccaggcccgtggttcctccactgccacattgaccctcacctcgacgccggcatggctgtagtcatggccgaggacactcccgacgtcgccgctacgaacccggtcccgcaagcatggtcggacttgtgccccatctatgatgcacttgaccccagcgacctctga

SEQ ID NO: 34 - DNA, 1491 bp, Artificial Sequence
  Engineered laccase F392T-F396I- F460M-D263V
agcattgggccagtcgcagacctcaccatctccaacggtgctgtcagtcccgatggtttctctcggcaggccatcctggtcaacgacgtcttccccagtcccctcattacggggaacaagggtgatcgtttccaactcaatgtcatcgacaacatgaccaaccacaccatgttgaagtccaccagtatccattggcacggcttcttccagcacggcaccaactgggccgacggccccgccttcgtgaaccagtgcccgatttctaccgggcatgcgttcctttacgacttccaggtccctgaccaagctggtactttctggtaccacagtcacttgtccactcaatactgtgacggtctcaggggtccgattgttgtctatgaccctcaagatccccacaagagcctttacgatgttgatgacgactccactgtaatcactctcgcggattggtaccacttggctgccaaagtcggcccggcggccccgactgccgatgctactcttatcaacggcctcggtcgcagcatcaacacgctcaacgccgatttggctgtcatcacggtcacgaagggcaagcgctatcgcttccgcctggtgtcgctgtcatgcgacccgtcttacacgttcagcattgatggtcactctctgaccgtcatcgaggcggacggcgtgaatctcaagccccagactgtcgactccatccagatcttccctgcccagcgatactcgtttgtgctcaacgcagatcaggatgtggacaactactggatccgtgcccttcccgtttccgggaccaggaacttcgacggcggcgttaactccgccatccttcgctacgaaggtgctgcgcccgttgagcccaccacgagccagacgccgtcgacgcagcctttggtggagtccgccctgaccactctcgaaggcaccgctgcgcccggcaacccgacccctggcggtgtcgacctggctctcaacatggctttcggctttgccggcggcaggttcaccatcaacggcgcgagcttcaccccgcccaccgtccccgtcctcctgcagatcctgagcggcgcgcagtcggcgcaggacctcctcccctctggaagtgtatactcgctccctgcgaacgcggacattgagatctccctccccgccacctccgccgcccccggcacuccgcaccccatccacttgcacgggcacaccttcgccgtcgtgcgcagcgccggctcgtcgacgtacaactacgcgaacccggtctaccgcgacgtcgtcaacacgggctcgcccggggacaacgtcacgatccggttcaggacggacaacccaggcccgtggttcctccactgccacattgaccctcacctcgacgccggcatggctgtagtcatggccgaggacactcccgacgtcgccgctacgaacccggtcccgcaagcatggtcggacttgtgccccatctatgatgcacttgaccccagcgacctctga

SEQ ID NO: 35 - DNA, 1491 bp, Artificial Sequence
  Engineered laccase F392T-F396I- F460M-D263V-A458L
agcattgggccagtcgcagacctcaccatctccaacggtgctgtcagtcccgatggtttctctcggcaggccatcctggtcaacgacgtcttccccagtcccctcattacggggaacaagggtgatcgtttccaactcaatgtcatcgacaacatgaccaaccacaccatgttgaagtccaccagtatccattggcacggcttcttccagcacggcaccaactgggccgacggccccgccttcgtgaaccagtgcccgatttctaccgggcatgcgttcctttacgacttccaggtccctgaccaagctggtactttctggtaccacagtcacttgtccactcaatactgtgacggtctcaggggtccgattgttgtctatgaccctcaagatccccacaagagcctttacgatgttgatgacgactccactgtaatcactctcgcggattggtaccacttggctgccaaagtcggcccggcggccccgactgccgatgctactcttatcaacggcctcggtcgcagcatcaacacgctcaacgccgatttggctgtcatcacggtcacgaagggcaagcgctatcgcttccgcctggtgtcgctgtcatgcgacccgtcttacacgttcagcattgatggtcactctctgaccgtcatcgaggcggacggcgtgaatctcaagccccagactgtcgactccatccagatcttccctgcccagcgatactcgtttgtgctcaacgcagatcaggatgtggacaactactggatccgtgcccttcccgtttccgggaccaggaacttcgacggcggcgttaactccgccatccttcgctacgaaggtgctgcgcccgttgagcccaccacgagccagacgccgtcgacgcagcctttggtggagtccgccctgaccactctcgaaggcaccgctgcgcccggcaacccgacccctggcggtgtcgacctggctctcaacatggctttcggctttgccggcggcaggttcaccatcaacggcgcgagcttcaccccgcccaccgtccccgtcctcctgcagatcctgagcggcgcgcagtcggcgcaggacctcctcccctctggaagtgtatactcgctccctgcgaacgcggacattgagatctccctccccgccacctccgccgcccccggcacuccgcaccccatccacttgcacgggcacaccttcgccgtcgtgcgcagcgccggctcgtcgacgtacaactacgcgaacccggtctaccgcgacgtcgtcaacacgggctcgcccggggacaacgtcacgatccggttcaggacggacaacccaggcccgtggttcctccactgccacattgaccctcacctcgacctaggcatggctgtagtcatggccgaggacactcccgacgtcgccgctacgaacccggtcccgcaagcatggtcggacttgtgccccatctatgatgcacttgaccccagcgacctctga

SEQ ID NO: 36 - DNA, 1491 bp, Artificial Sequence
  Engineered laccase F392T-F396I- F460M-D263V-A458L-V424T-S429T-D441N
agcattgggccagtcgcagacctcaccatctccaacggtgctgtcagtcccgatggtttctctcggcaggccatcctggtcaacgacgtcttccccagtcccctcattacggggaacaagggtgatcgtttccaactcaatgtcatcgacaacatgaccaaccacaccatgttgaagtccaccagtatccattggcacggcttcttccagcacggcaccaactgggccgacggccccgccttcgtgaaccagtgcccgatttctaccgggcatgcgttcctttacgacttccaggtccctgaccaagctggtactttctggtaccacagtcacttgtccactcaatactgtgacggtctcaggggtccgattgttgtctatgaccctcaagatccccacaagagcctttacgatgttgatgacgactccactgtaatcactctcgcggattggtaccacttggctgccaaagtcggcccggcggccccgactgccgatgctactcttatcaacggcctcggtcgcagcatcaacacgctcaacgccgatttggctgtcatcacggtcacgaagggcaagcgctatcgcttccgcctggtgtcgctgtcatgcgacccgtcttacacgttcagcattgatggtcactctctgaccgtcatcgaggcggacggcgtgaatctcaagccccagactgtcgactccatccagatcttccctgcccagcgatactcgtttgtgctcaacgcagatcaggatgtggacaactactggatccgtgcccttcccgtttccgggaccaggaacttcgacggcggcgttaactccgccatccttcgctacgaaggtgctgcgcccgttgagcccaccacgagccagacgccgtcgacgcagcctttggtggagtccgccctgaccactctcgaaggcaccgctgcgcccggcaacccgacccctggcggtgtcgacctggctctcaacatggctttcggctttgccggcggcaggttcaccatcaacggcgcgagcttcaccccgcccaccgtccccgtcctcctgcagatcctgagcggcgcgcagtcggcgcaggacctcctcccctctggaagtgtatactcgctccctgcgaacgcggacattgagatctccctccccgccacctccgccgcccccggcacuccgcaccccatccacttgcacgggcacaccttcgccgtcgtgcgcagcgccggctcgtcgacgtacaactacgcgaacccggtctaccgcgacactgtcaacacgggcactcccggggacaacgtcacgatccggttcaggacgaataacccaggcccgtggttcctccactgccacattgaccctcacctcgacctaggcatggctgtagtcatggccgaggacactcccgacgtcgccgctacgaacccggtcccgcaagcatggtcggacttgtgccccatctatgatgcacttgaccccagcgacctctga

SEQ ID NO: 37 - DNA, 1491 bp, Artificial Sequence
  Engineered laccase F392T-F396I- F460M-D263A
agcattgggccagtcgcagacctcaccatctccaacggtgctgtcagtcccgatggtttctctcggcaggccatcctggtcaacgacgtcttccccagtcccctcattacggggaacaagggtgatcgtttccaactcaatgtcatcgacaacatgaccaaccacaccatgttgaagtccaccagtatccattggcacggcttcttccagcacggcaccaactgggccgacggccccgccttcgtgaaccagtgcccgatttctaccgggcatgcgttcctttacgacttccaggtccctgaccaagctggtactttctggtaccacagtcacttgtccactcaatactgtgacggtctcaggggtccgattgttgtctatgaccctcaagatccccacaagagcctttacgatgttgatgacgactccactgtaatcactctcgcggattggtaccacttggctgccaaagtcggcccggcggccccgactgccgatgctactcttatcaacggcctcggtcgcagcatcaacacgctcaacgccgatttggctgtcatcacggtcacgaagggcaagcgctatcgcttccgcctggtgtcgctgtcatgcgacccgtcttacacgttcagcattgatggtcactctctgaccgtcatcgaggcggacggcgtgaatctcaagccccagactgtcgactccatccagatcttccctgcccagcgatactcgtttgtgctcaacgcagatcaggatgtggacaactactggatccgtgcccttcccgcutccgggaccaggaacttcgacggcggcgttaactccgccatccttcgctacgaaggtgctgcgcccgttgagcccaccacgagccagacgccgtcgacgcagcctttggtggagtccgccctgaccactctcgaaggcaccgctgcgcccggcaacccgacccctggcggtgtcgacctggctctcaacatggctttcggctttgccggcggcaggttcaccatcaacggcgcgagcttcaccccgcccaccgtccccgtcctcctgcagatcctgagcggcgcgcagtcggcgcaggacctcctcccctctggaagtgtatactcgctccctgcgaacgcggacattgagatctccctccccgccacctccgccgcccccggcacuccgcaccccatccacttgcacgggcacaccttcgccgtcgtgcgcagcgccggctcgtcgacgtacaactacgcgaacccggtctaccgcgacgtcgtcaacacgggctcgcccggggacaacgtcacgatccggttcaggacggacaacccaggcccgtggttcctccactgccacattgaccctcacctcgacgccggcatggctgtagtcatggccgaggacactcccgacgtcgccgctacgaacccggtcccgcaagcatggtcggacttgtgccccatctatgatgcacttgaccccagcgacctctga

SEQ ID NO: 38 - DNA, 1491 bp, Artificial Sequence
  Engineered laccase F392T-F396I- F460M-D263A-A458L
agcattgggccagtcgcagacctcaccatctccaacggtgctgtcagtcccgatggtttctctcggcaggccatcctggtcaacgacgtcttccccagtcccctcattacggggaacaagggtgatcgtttccaactcaatgtcatcgacaacatgaccaaccacaccatgttgaagtccaccagtatccattggcacggcttcttccagcacggcaccaactgggccgacggccccgccttcgtgaaccagtgcccgatttctaccgggcatgcgttcctttacgacttccaggtccctgaccaagctggtactttctggtaccacagtcacttgtccactcaatactgtgacggtctcaggggtccgattgttgtctatgaccctcaagatccccacaagagcctttacgatgttgatgacgactccactgtaatcactctcgcggattggtaccacttggctgccaaagtcggcccggcggccccgactgccgatgctactcttatcaacggcctcggtcgcagcatcaacacgctcaacgccgatttggctgtcatcacggtcacgaagggcaagcgctatcgcttccgcctggtgtcgctgtcatgcgacccgtcttacacgttcagcattgatggtcactctctgaccgtcatcgaggcggacggcgtgaatctcaagccccagactgtcgactccatccagatcttccctgcccagcgatactcgtttgtgctcaacgcagatcaggatgtggacaactactggatccgtgcccttcccgcutccgggaccaggaacttcgacggcggcgttaactccgccatccttcgctacgaaggtgctgcgcccgttgagcccaccacgagccagacgccgtcgacgcagcctttggtggagtccgccctgaccactctcgaaggcaccgctgcgcccggcaacccgacccctggcggtgtcgacctggctctcaacatggctttcggctttgccggcggcaggttcaccatcaacggcgcgagcttcaccccgcccaccgtccccgtcctcctgcagatcctgagcggcgcgcagtcggcgcaggacctcctcccctctggaagtgtatactcgctccctgcgaacgcggacattgagatctccctccccgccacctccgccgcccccggcacuccgcaccccatccacttgcacgggcacaccttcgccgtcgtgcgcagcgccggctcgtcgacgtacaactacgcgaacccggtctaccgcgacgtcgtcaacacgggctcgcccggggacaacgtcacgatccggttcaggacggacaacccaggcccgtggttcctccactgccacattgaccctcacctcgacctaggcatggctgtagtcatggccgaggacactcccgacgtcgccgctacgaacccggtcccgcaagcatggtcggacttgtgccccatctatgatgcacttgaccccagcgacctctga

SEQ ID NO: 39 - DNA, 1491 bp, Artificial Sequence
  Engineered laccase F392T-F396I- F460M-D263A-A458L-V424T-S429T-D441N
agcattgggccagtcgcagacctcaccatctccaacggtgctgtcagtcccgatggtttctctcggcaggccatcctggtcaacgacgtcttccccagtcccctcattacggggaacaagggtgatcgtttccaactcaatgtcatcgacaacatgaccaaccacaccatgttgaagtccaccagtatccattggcacggcttcttccagcacggcaccaactgggccgacggccccgccttcgtgaaccagtgcccgatttctaccgggcatgcgttcctttacgacttccaggtccctgaccaagctggtactttctggtaccacagtcacttgtccactcaatactgtgacggtctcaggggtccgattgttgtctatgaccctcaagatccccacaagagcctttacgatgttgatgacgactccactgtaatcactctcgcggattggtaccacttggctgccaaagtcggcccggcggccccgactgccgatgctactcttatcaacggcctcggtcgcagcatcaacacgctcaacgccgatttggctgtcatcacggtcacgaagggcaagcgctatcgcttccgcctggtgtcgctgtcatgcgacccgtcttacacgttcagcattgatggtcactctctgaccgtcatcgaggcggacggcgtgaatctcaagccccagactgtcgactccatccagatcttccctgcccagcgatactcgtttgtgctcaacgcagatcaggatgtggacaactactggatccgtgcccttcccgcutccgggaccaggaacttcgacggcggcgttaactccgccatccttcgctacgaaggtgctgcgcccgttgagcccaccacgagccagacgccgtcgacgcagcctttggtggagtccgccctgaccactctcgaaggcaccgctgcgcccggcaacccgacccctggcggtgtcgacctggctctcaacatggctttcggctttgccggcggcaggttcaccatcaacggcgcgagcttcaccccgcccaccgtccccgtcctcctgcagatcctgagcggcgcgcagtcggcgcaggacctcctcccctctggaagtgtatactcgctccctgcgaacgcggacattgagatctccctccccgccacctccgccgcccccggcacuccgcaccccatccacttgcacgggcacaccttcgccgtcgtgcgcagcgccggctcgtcgacgtacaactacgcgaacccggtctaccgcgacactgtcaacacgggcactcccggggacaacgtcacgatccggttcaggacgaataacccaggcccgtggttcctccactgccacattgaccctcacctcgacctaggcatggctgtagtcatggccgaggacactcccgacgtcgccgctacgaacccggtcccgcaagcatggtcggacttgtgccccatctatgatgcacttgaccccagcgacctctga

SEQ ID NO: 40 - DNA, 1491 bp, Artificial Sequence
  Engineered laccase F392T-F396I- F460M-D263G
agcattgggccagtcgcagacctcaccatctccaacggtgctgtcagtcccgatggtttctctcggcaggccatcctggtcaacgacgtcttccccagtcccctcattacggggaacaagggtgatcgtttccaactcaatgtcatcgacaacatgaccaaccacaccatgttgaagtccaccagtatccattggcacggcttcttccagcacggcaccaactgggccgacggccccgccttcgtgaaccagtgcccgatttctaccgggcatgcgttcctttacgacttccaggtccctgaccaagctggtactttctggtaccacagtcacttgtccactcaatactgtgacggtctcaggggtccgattgttgtctatgaccctcaagatccccacaagagcctttacgatgttgatgacgactccactgtaatcactctcgcggattggtaccacttggctgccaaagtcggcccggcggccccgactgccgatgctactcttatcaacggcctcggtcgcagcatcaacacgctcaacgccgatttggctgtcatcacggtcacgaagggcaagcgctatcgcttccgcctggtgtcgctgtcatgcgacccgtcttacacgttcagcattgatggtcactctctgaccgtcatcgaggcggacggcgtgaatctcaagccccagactgtcgactccatccagatcttccctgcccagcgatactcgtttgtgctcaacgcagatcaggatgtggacaactactggatccgtgcccttcccggutccgggaccaggaacttcgacggcggcgttaactccgccatccttcgctacgaaggtgctgcgcccgttgagcccaccacgagccagacgccgtcgacgcagcctttggtggagtccgccctgaccactctcgaaggcaccgctgcgcccggcaacccgacccctggcggtgtcgacctggctctcaacatggctttcggctttgccggcggcaggttcaccatcaacggcgcgagcttcaccccgcccaccgtccccgtcctcctgcagatcctgagcggcgcgcagtcggcgcaggacctcctcccctctggaagtgtatactcgctccctgcgaacgcggacattgagatctccctccccgccacctccgccgcccccggcacuccgcaccccatccacttgcacgggcacaccttcgccgtcgtgcgcagcgccggctcgtcgacgtacaactacgcgaacccggtctaccgcgacgtcgtcaacacgggctcgcccggggacaacgtcacgatccggttcaggacggacaacccaggcccgtggttcctccactgccacattgaccctcacctcgacgccggcatggctgtagtcatggccgaggacactcccgacgtcgccgctacgaacccggtcccgcaagcatggtcggacttgtgccccatctatgatgcacttgaccccagcgacctctga

SEQ ID NO: 41 - DNA, 1491 bp, Artificial Sequence
  Engineered laccase F392T-F396I- F460M-D263G-A58L
agcattgggccagtcgcagacctcaccatctccaacggtgctgtcagtcccgatggtttctctcggcaggccatcctggtcaacgacgtcttccccagtcccctcattacggggaacaagggtgatcgtttccaactcaatgtcatcgacaacatgaccaaccacaccatgttgaagtccaccagtatccattggcacggcttcttccagcacggcaccaactgggccgacggccccgccttcgtgaaccagtgcccgatttctaccgggcatgcgttcctttacgacttccaggtccctgaccaagctggtactttctggtaccacagtcacttgtccactcaatactgtgacggtctcaggggtccgattgttgtctatgaccctcaagatccccacaagagcctttacgatgttgatgacgactccactgtaatcactctcgcggattggtaccacttggctgccaaagtcggcccggcggccccgactgccgatgctactcttatcaacggcctcggtcgcagcatcaacacgctcaacgccgatttggctgtcatcacggtcacgaagggcaagcgctatcgcttccgcctggtgtcgctgtcatgcgacccgtcttacacgttcagcattgatggtcactctctgaccgtcatcgaggcggacggcgtgaatctcaagccccagactgtcgactccatccagatcttccctgcccagcgatactcgtttgtgctcaacgcagatcaggatgtggacaactactggatccgtgcccttcccggutccgggaccaggaacttcgacggcggcgttaactccgccatccttcgctacgaaggtgctgcgcccgttgagcccaccacgagccagacgccgtcgacgcagcctttggtggagtccgccctgaccactctcgaaggcaccgctgcgcccggcaacccgacccctggcggtgtcgacctggctctcaacatggctttcggctttgccggcggcaggttcaccatcaacggcgcgagcttcaccccgcccaccgtccccgtcctcctgcagatcctgagcggcgcgcagtcggcgcaggacctcctcccctctggaagtgtatactcgctccctgcgaacgcggacattgagatctccctccccgccacctccgccgcccccggcacuccgcaccccatccacttgcacgggcacaccttcgccgtcgtgcgcagcgccggctcgtcgacgtacaactacgcgaacccggtctaccgcgacgtcgtcaacacgggctcgcccggggacaacgtcacgatccggttcaggacggacaacccaggcccgtggttcctccactgccacattgaccctcacctcgacctaggcatggctgtagtcatggccgaggacactcccgacgtcgccgctacgaacccggtcccgcaagcatggtcggacttgtgccccatctatgatgcacttgaccccagcgacctctga

SEQ ID NO: 42 - DNA, 1491 bp, Artificial Sequence
  Engineered laccase F392T-F396I- F460M-D263G-A58L-V424T-S429T-D441N
agcattgggccagtcgcagacctcaccatctccaacggtgctgtcagtcccgatggtttctctcggcaggccatcctggtcaacgacgtcttccccagtcccctcattacggggaacaagggtgatcgtttccaactcaatgtcatcgacaacatgaccaaccacaccatgttgaagtccaccagtatccattggcacggcttcttccagcacggcaccaactgggccgacggccccgccttcgtgaaccagtgcccgatttctaccgggcatgcgttcctttacgacttccaggtccctgaccaagctggtactttctggtaccacagtcacttgtccactcaatactgtgacggtctcaggggtccgattgttgtctatgaccctcaagatccccacaagagcctttacgatgttgatgacgactccactgtaatcactctcgcggattggtaccacttggctgccaaagtcggcccggcggccccgactgccgatgctactcttatcaacggcctcggtcgcagcatcaacacgctcaacgccgatttggctgtcatcacggtcacgaagggcaagcgctatcgcttccgcctggtgtcgctgtcatgcgacccgtcttacacgttcagcattgatggtcactctctgaccgtcatcgaggcggacggcgtgaatctcaagccccagactgtcgactccatccagatcttccctgcccagcgatactcgtttgtgctcaacgcagatcaggatgtggacaactactggatccgtgcccttcccggutccgggaccaggaacttcgacggcggcgttaactccgccatccttcgctacgaaggtgctgcgcccgttgagcccaccacgagccagacgccgtcgacgcagcctttggtggagtccgccctgaccactctcgaaggcaccgctgcgcccggcaacccgacccctggcggtgtcgacctggctctcaacatggctttcggctttgccggcggcaggttcaccatcaacggcgcgagcttcaccccgcccaccgtccccgtcctcctgcagatcctgagcggcgcgcagtcggcgcaggacctcctcccctctggaagtgtatactcgctccctgcgaacgcggacattgagatctccctccccgccacctccgccgcccccggcacuccgcaccccatccacttgcacgggcacaccttcgccgtcgtgcgcagcgccggctcgtcgacgtacaactacgcgaacccggtctaccgcgacactgtcaacacgggcactcccggggacaacgtcacgatccggttcaggacgaataacccaggcccgtggttcctccactgccacattgaccctcacctcgacctaggcatggctgtagtcatggccgaggacactcccgacgtcgccgctacgaacccggtcccgcaagcatggtcggacttgtgccccatctatgatgcacttgaccccagcgacctctga

SEQ ID NO: 43 - DNA, 273 bp, Artificial Sequence
  Signal peptide RY2-L4
atgagatttccttcaatttttactgatgttttattcgcagcatcctccgcattagctactccagtcaacactacaacagaagatgaaacggcacatattccggctgaagctgtcatcggttactcagatttagaaggggattccgatgttgctgttctgccattttccaacggcacaaataacagattattgtttataaatactactattgccagcattgctgctaaagaagaaggggtatctctcgagaaaagagagactgaagctgaattc

SEQ ID NO: 44 - DNA, 273 bp, Artificial Sequence
  Signal peptide L5
atgagatttccttcaatttttactgatgttttattcgcagcatcctccgcattagctactccagtcaacactacaacagaagatgaaacggcacaaattccggctgaagctgtcatcggttactcagatttagaaggggatttcgatgttgctgttttgccattttccaacagcacaaataacggtttattgtttataaatactactattgccagcattgctgctaaagaagaaggggtatctctcgagaaaagaactaatgaagctgaattc

SEQ ID NO: 45 - DNA, 1491 bp, Artificial Sequence
  Engineered laccase F392T-F396I-F460M-D263A
agcattgggccagtcgcagacctcaccatctccaacggtgctgtcagtcccgatggtttctctcggcaggccatcctggtcaacgacgtcttccccagtcccctcattacggggaacaagggtgatcgtttccaactcaatgtcatcgacaacatgaccaaccacaccatgttgaagtccaccagtatccattggcacggcttcttccagcacggcaccaactgggccgacggccccgccttcgtgaaccagtgcccgatttctaccgggcatgcgttcctttacgacttccaggtccctgaccaagctggtactttctggtaccacagtcacttgtccactcaatactgtgacggtctcaggggtccgattgttgtctatgaccctcaagatccccacaagagcctttacgatgttgatgacgactccactgtaatcactctcgcggattggtaccacttggctgccaaagtcggcccggcggccccgactgccgatgctactcttatcaacggcctcggtcgcagcatcaacacgctcaacgccgatttggctgtcatcacggtcacgaagggcaagcgctatcgcttccgcctggtgtcgctgtcatgcgacccgtcttacacgttcagcattgatggtcactctctgaccgtcatcgaggcggacggcgtgaatctcaagccccagactgtcgactccatccagatcttccctgcccagcgatactcgtttgtgctcaacgcagatcaggatgtggacaactactggatccgtgcccttcccgcutccgggaccaggaacttcgacggcggcgttaactccgccatccttcgctacgaaggtgctgcgcccgttgagcccaccacgagccagacgccgtcgacgcagcctttggtggagtccgccctgaccactctcgaaggcaccgctgcgcccggcaacccgacccctggcggtgtcgacctggctctcaacatggctttcggctttgccggcggcaggttcaccatcaacggcgcgagcttcaccccgcccaccgtccccgtcctcctgcagatcctgagcggcgcgcagtcggcgcaggacctcctcccctctggaagtgtatactcgctccctgcgaacgcggacattgagatctccctccccgccacctccgccgcccccggcaatccgcaccccatccacttgcacgggcacaccttcgccgtcgtgcgcagcgccggctcgtcgacgtacaactacgcgaacccggtctaccgcgacgtcgtcaacacgggctcgcccggggacaacgtcacgatccggttcaggacggacaacccaggcccgtggttcctccactgccacattgaccctcacctcgacgccggcatggctgtagtcatggccgaggacactcccgacgtcgccgctacgaacccggtcccgcaagcatggtcggacttgtgccccatctatgatgcacttgaccccagcgacctctga

SEQ ID NO: 46 - DNA, 1491 bp, Artificial Sequence
  Engineered laccase F392T-F396I-F460M-D263A-A458L
agcattgggccagtcgcagacctcaccatctccaacggtgctgtcagtcccgatggtttctctcggcaggccatcctggtcaacgacgtcttccccagtcccctcattacggggaacaagggtgatcgtttccaactcaatgtcatcgacaacatgaccaaccacaccatgttgaagtccaccagtatccattggcacggcttcttccagcacggcaccaactgggccgacggccccgccttcgtgaaccagtgcccgatttctaccgggcatgcgttcctttacgacttccaggtccctgaccaagctggtactttctggtaccacagtcacttgtccactcaatactgtgacggtctcaggggtccgattgttgtctatgaccctcaagatccccacaagagcctttacgatgttgatgacgactccactgtaatcactctcgcggattggtaccacttggctgccaaagtcggcccggcggccccgactgccgatgctactcttatcaacggcctcggtcgcagcatcaacacgctcaacgccgatttggctgtcatcacggtcacgaagggcaagcgctatcgcttccgcctggtgtcgctgtcatgcgacccgtcttacacgttcagcattgatggtcactctctgaccgtcatcgaggcggacggcgtgaatctcaagccccagactgtcgactccatccagatcttccctgcccagcgatactcgtttgtgctcaacgcagatcaggatgtggacaactactggatccgtgcccttcccgcutccgggaccaggaacttcgacggcggcgttaactccgccatccttcgctacgaaggtgctgcgcccgttgagcccaccacgagccagacgccgtcgacgcagcctttggtggagtccgccctgaccactctcgaaggcaccgctgcgcccggcaacccgacccctggcggtgtcgacctggctctcaacatggctttcggctttgccggcggcaggttcaccatcaacggcgcgagcttcaccccgcccaccgtccccgtcctcctgcagatcctgagcggcgcgcagtcggcgcaggacctcctcccctctggaagtgtatactcgctccctgcgaacgcggacattgagatctccctccccgccacctccgccgcccccggcaatccgcaccccatccacttgcacgggcacaccttcgccgtcgtgcgcagcgccggctcgtcgacgtacaactacgcgaacccggtctaccgcgacgtcgtcaacacgggctcgcccggggacaacgtcacgatccggttcaggacggacaacccaggcccgtggttcctccactgccacattgaccctcacctcgacctaggcatggctgtagtcatggccgaggacactcccgacgtcgccgctacgaacccggtcccgcaagcatggtcggacttgtgccccatctatgatgcacttgaccccagcgacctctga

SEQ ID NO: 47 - DNA, 1491 bp, Artificial Sequence
  Engineered laccase F392N-F396I-F460M-D263A-A458L-V424T-S429T-D441N
agcattgggccagtcgcagacctcaccatctccaacggtgctgtcagtcccgatggtttctctcggcaggccatcctggtcaacgacgtcttccccagtcccctcattacggggaacaagggtgatcgtttccaactcaatgtcatcgacaacatgaccaaccacaccatgttgaagtccaccagtatccattggcacggcttcttccagcacggcaccaactgggccgacggccccgccttcgtgaaccagtgcccgatttctaccgggcatgcgttcctttacgacttccaggtccctgaccaagctggtactttctggtaccacagtcacttgtccactcaatactgtgacggtctcaggggtccgattgttgtctatgaccctcaagatccccacaagagcctttacgatgttgatgacgactccactgtaatcactctcgcggattggtaccacttggctgccaaagtcggcccggcggccccgactgccgatgctactcttatcaacggcctcggtcgcagcatcaacacgctcaacgccgatttggctgtcatcacggtcacgaagggcaagcgctatcgcttccgcctggtgtcgctgtcatgcgacccgtcttacacgttcagcattgatggtcactctctgaccgtcatcgaggcggacggcgtgaatctcaagccccagactgtcgactccatccagatcttccctgcccagcgatactcgtttgtgctcaacgcagatcaggatgtggacaactactggatccgtgcccttcccgcutccgggaccaggaacttcgacggcggcgttaactccgccatccttcgctacgaaggtgctgcgcccgttgagcccaccacgagccagacgccgtcgacgcagcctttggtggagtccgccctgaccactctcgaaggcaccgctgcgcccggcaacccgacccctggcggtgtcgacctggctctcaacatggctttcggctttgccggcggcaggttcaccatcaacggcgcgagcttcaccccgcccaccgtccccgtcctcctgcagatcctgagcggcgcgcagtcggcgcaggacctcctcccctctggaagtgtatactcgctccctgcgaacgcggacattgagatctccctccccgccacctccgccgcccccggcaatccgcaccccatccacttgcacgggcacaccttcgccgtcgtgcgcagcgccggctcgtcgacgtacaactacgcgaacccggtctaccgcgacactgtcaacacgggcactcccggggacaacgtcacgatccggttcaggacgaataacccaggcccgtggttcctccactgccacattgaccctcacctcgacctaggcatggctgtagtcatggccgaggacactcccgacgtcgccgctacgaacccggtcccgcaagcatggtcggacttgtgccccatctatgatgcacttgaccccagcgacctctga

SEQ ID NO: 48 - DNA, 1491 bp, Artificial Sequence
  Engineered laccase F392N-F396I-F460M-D263G
agcattgggccagtcgcagacctcaccatctccaacggtgctgtcagtcccgatggtttctctcggcaggccatcctggtcaacgacgtcttccccagtcccctcattacggggaacaagggtgatcgtttccaactcaatgtcatcgacaacatgaccaaccacaccatgttgaagtccaccagtatccattggcacggcttcttccagcacggcaccaactgggccgacggccccgccttcgtgaaccagtgcccgatttctaccgggcatgcgttcctttacgacttccaggtccctgaccaagctggtactttctggtaccacagtcacttgtccactcaatactgtgacggtctcaggggtccgattgttgtctatgaccctcaagatccccacaagagcctttacgatgttgatgacgactccactgtaatcactctcgcggattggtaccacttggctgccaaagtcggcccggcggccccgactgccgatgctactcttatcaacggcctcggtcgcagcatcaacacgctcaacgccgatttggctgtcatcacggtcacgaagggcaagcgctatcgcttccgcctggtgtcgctgtcatgcgacccgtcttacacgttcagcattgatggtcactctctgaccgtcatcgaggcggacggcgtgaatctcaagccccagactgtcgactccatccagatcttccctgcccagcgatactcgtttgtgctcaacgcagatcaggatgtggacaactactggatccgtgcccttcccggutccgggaccaggaacttcgacggcggcgttaactccgccatccttcgctacgaaggtgctgcgcccgttgagcccaccacgagccagacgccgtcgacgcagcctttggtggagtccgccctgaccactctcgaaggcaccgctgcgcccggcaacccgacccctggcggtgtcgacctggctctcaacatggctttcggctttgccggcggcaggttcaccatcaacggcgcgagcttcaccccgcccaccgtccccgtcctcctgcagatcctgagcggcgcgcagtcggcgcaggacctcctcccctctggaagtgtatactcgctccctgcgaacgcggacattgagatctccctccccgccacctccgccgcccccggcaatccgcaccccatccacttgcacgggcacaccttcgccgtcgtgcgcagcgccggctcgtcgacgtacaactacgcgaacccggtctaccgcgacgtcgtcaacacgggctcgcccggggacaacgtcacgatccggttcaggacggacaacccaggcccgtggttcctccactgccacattgaccctcacctcgacgccggcatggctgtagtcatggccgaggacactcccgacgtcgccgctacgaacccggtcccgcaagcatggtcggacttgtgccccatctatgatgcacttgaccccagcgacctctga

SEQ ID NO: 49 - DNA, 1491 bp, Artificial Sequence
  Engineered laccase F392N-F396I-F460M-D263G-A458L
agcattgggccagtcgcagacctcaccatctccaacggtgctgtcagtcccgatggtttctctcggcaggccatcctggtcaacgacgtcttccccagtcccctcattacggggaacaagggtgatcgtttccaactcaatgtcatcgacaacatgaccaaccacaccatgttgaagtccaccagtatccattggcacggcttcttccagcacggcaccaactgggccgacggccccgccttcgtgaaccagtgcccgatttctaccgggcatgcgttcctttacgacttccaggtccctgaccaagctggtactttctggtaccacagtcacttgtccactcaatactgtgacggtctcaggggtccgattgttgtctatgaccctcaagatccccacaagagcctttacgatgttgatgacgactccactgtaatcactctcgcggattggtaccacttggctgccaaagtcggcccggcggccccgactgccgatgctactcttatcaacggcctcggtcgcagcatcaacacgctcaacgccgatttggctgtcatcacggtcacgaagggcaagcgctatcgcttccgcctggtgtcgctgtcatgcgacccgtcttacacgttcagcattgatggtcactctctgaccgtcatcgaggcggacggcgtgaatctcaagccccagactgtcgactccatccagatcttccctgcccagcgatactcgtttgtgctcaacgcagatcaggatgtggacaactactggatccgtgcccttcccggutccgggaccaggaacttcgacggcggcgttaactccgccatccttcgctacgaaggtgctgcgcccgttgagcccaccacgagccagacgccgtcgacgcagcctttggtggagtccgccctgaccactctcgaaggcaccgctgcgcccggcaacccgacccctggcggtgtcgacctggctctcaacatggctttcggctttgccggcggcaggttcaccatcaacggcgcgagcttcaccccgcccaccgtccccgtcctcctgcagatcctgagcggcgcgcagtcggcgcaggacctcctcccctctggaagtgtatactcgctccctgcgaacgcggacattgagatctccctccccgccacctccgccgcccccggcaatccgcaccccatccacttgcacgggcacaccttcgccgtcgtgcgcagcgccggctcgtcgacgtacaactacgcgaacccggtctaccgcgacgtcgtcaacacgggctcgcccggggacaacgtcacgatccggttcaggacggacaacccaggcccgtggttcctccactgccacattgaccctcacctcgacctaggcatggctgtagtcatggccgaggacactcccgacgtcgccgctacgaacccggtcccgcaagcatggtcggacttgtgccccatctatgatgcacttgaccccagcgacctctga

SEQ ID NO: 50 - DNA, 1491 bp, Artificial Sequence
  Engineered laccase F392N-F396I-F460M-D263G-A458L-V424T-S429T-D441N
agcattgggccagtcgcagacctcaccatctccaacggtgctgtcagtcccgatggtttctctcggcaggccatcctggtcaacgacgtcttccccagtcccctcattacggggaacaagggtgatcgtttccaactcaatgtcatcgacaacatgaccaaccacaccatgttgaagtccaccagtatccattggcacggcttcttccagcacggcaccaactgggccgacggccccgccttcgtgaaccagtgcccgatttctaccgggcatgcgttcctttacgacttccaggtccctgaccaagctggtactttctggtaccacagtcacttgtccactcaatactgtgacggtctcaggggtccgattgttgtctatgaccctcaagatccccacaagagcctttacgatgttgatgacgactccactgtaatcactctcgcggattggtaccacttggctgccaaagtcggcccggcggccccgactgccgatgctactcttatcaacggcctcggtcgcagcatcaacacgctcaacgccgatttggctgtcatcacggtcacgaagggcaagcgctatcgcttccgcctggtgtcgctgtcatgcgacccgtcttacacgttcagcattgatggtcactctctgaccgtcatcgaggcggacggcgtgaatctcaagccccagactgtcgactccatccagatcttccctgcccagcgatactcgtttgtgctcaacgcagatcaggatgtggacaactactggatccgtgcccttcccggutccgggaccaggaacttcgacggcggcgttaactccgccatccttcgctacgaaggtgctgcgcccgttgagcccaccacgagccagacgccgtcgacgcagcctttggtggagtccgccctgaccactctcgaaggcaccgctgcgcccggcaacccgacccctggcggtgtcgacctggctctcaacatggctttcggctttgccggcggcaggttcaccatcaacggcgcgagcttcaccccgcccaccgtccccgtcctcctgcagatcctgagcggcgcgcagtcggcgcaggacctcctcccctctggaagtgtatactcgctccctgcgaacgcggacattgagatctccctccccgccacctccgccgcccccggcaatccgcaccccatccacttgcacgggcacaccttcgccgtcgtgcgcagcgccggctcgtcgacgtacaactacgcgaacccggtctaccgcgacactgtcaacacgggcactcccggggacaacgtcacgatccggttcaggacgaataacccaggcccgtggttcctccactgccacattgaccctcacctcgacctaggcatggctgtagtcatggccgaggacactcccgacgtcgccgctacgaacccggtcccgcaagcatggtcggacttgtgccccatctatgatgcacttgaccccagcgacctctga

SEQ ID NO: 51 - protein, 496 aa, Artificial Sequence
  Engineered laccase F392N-F396I-L456M-A458T
SIGPVADLTISNGAVSPDGFSRQAILVNDVFPSPLITGNKGDRFQLNVIDNMTNHTMLKSTSIHWHGFFQHGTNWADGPAFVNQCPISTGHAFLYDFQVPDQAGTFWYHSHLSTQYCDGLRGPIVVYDPQDPHKSLYDVDDDSTVITLADWYHLAAKVGPAAPTADATLINGLGRSINTLNADLAVITVTKGKRYRFRLVSLSCDPSYTFSIDGHSLTVIEADGVNLKPQTVDSIQIFPAQRYSFVLNADQDVDNYWIRALPDSGTRNFDGGVNSAILRYEGAAPVEPTTSQTPSTQPLVESALTTLEGTAAPGNPTPGGVDLALNMAFGFAGGRFTINGASFTPPTVPVLLQILSGAQSAQDLLPSGSVYSLPANADIEISLPATSAAPGNPHPIHLHGHTFAVVRSAGSSTYNYANPVYRDVVNTGSPGDNVTIRFRTDNPGPWFLHCHIDPHMDTGFAVVMAEDTPDVAATNPVPQAWSDLCPIYDALDPSDL

SEQ ID NO: 52 - DNA, 1491 bp, Artificial Sequence
  Engineered laccase F392N-F396I-L456M-A458T
agcattgggccagtcgcagacctcaccatctccaacggtgctgtcagtcccgatggtttctctcggcaggccatcctggtcaacgacgtcttccccagtcccctcattacggggaacaagggtgatcgtttccaactcaatgtcatcgacaacatgaccaaccacaccatgttgaagtccaccagtatccattggcacggcttcttccagcacggcaccaactgggccgacggccccgccttcgtgaaccagtgcccgatttctaccgggcatgcgttcctttacgacttccaggtccctgaccaagctggtactttctggtaccacagtcacttgtccactcaatactgtgacggtctcaggggtccgattgttgtctatgaccctcaagatccccacaagagcctttacgatgttgatgacgactccactgtaatcactctcgcggattggtaccacttggctgccaaagtcggcccggcggccccgactgccgatgctactcttatcaacggcctcggtcgcagcatcaacacgctcaacgccgatttggctgtcatcacggtcacgaagggcaagcgctatcgcttccgcctggtgtcgctgtcatgcgacccgtcttacacgttcagcattgatggtcactctctgaccgtcatcgaggcggacggcgtgaatctcaagccccagactgtcgactccatccagatcttccctgcccagcgatactcgtttgtgctcaacgcagatcaggatgtggacaactactggatccgtgcccttcccgattccgggaccaggaacttcgacggcggcgttaactccgccatccttcgctacgaaggtgctgcgcccgttgagcccaccacgagccagacgccgtcgacgcagcctttggtggagtccgccctgaccactctcgaaggcaccgctgcgcccggcaacccgacccctggcggtgtcgacctggctctcaacatggctttcggctttgccggcggcaggttcaccatcaacggcgcgagcttcaccccgcccaccgtccccgtcctcctgcagatcctgagcggcgcgcagtcggcgcaggacctcctcccctctggaagtgtatactcgctccctgcgaacgcggacattgagatctccctccccgccacctccgccgcccccggcaatccgcaccccatccacttgcacgggcacaccttcgccgtcgtgcgcagcgccggctcgtcgacgtacaactacgcgaacccggtctaccgcgacgtcgtcaacacgggctcgcccggggacaacgtcacgatccggttcaggacggacaacccaggcccgtggttcctccactgccacattgaccctcacatggacacuggctttgctgtagtcatggccgaggacactcccgacgtcgccgctacgaacccggtcccgcaagcatggtcggacttgtgccccatctatgatgcacttgaccccagcgacctctga